European Patent Application EP 4 162 948 A1, published April 12, 2023. Title: Transcription Infidelity derived chimeric immunogens and uses thereof. Applicant: GENCLIS. The sequence listing filed with the application follows.

SEQUENCE LISTING (70 sequences)

SEQ ID NO: 1 - protein, 145 aa, Artificial Sequence
  canonical IL31
MKHHHHHHMSHMAPTHQLPPSDVRKIILELQPLSRGLLEDYQKKETGVPESNRTLLLCLTSDSQPPRLNSSAILPYFRAIRPLSDKNIIDKIIEQLDKLKFQHEPETEISVPADTFECKSFILTILQQFSACLESVFKSLNSGPQ

SEQ ID NO: 2 - protein, 178 aa, Artificial Sequence
  chimeric immunogen
MKHHHHHHMSHMAPTHQLPPSDVRKIILELQPLSRGLLEDYQKKETGVPESNRTLLLCLTSDSQPPRLNSSAILPYFRAIRPLSDKNIIDKIIEQLDKLKFQHEPETEISVPADTFECKSFILTILQQFSACLESVFKSLNSGPQLKIQKLQGKCSQPGMVGCSLTTWRTSMVLGRNI

SEQ ID NO: 3 - protein, 175 aa, Artificial Sequence
  chimeric immunogen
MKHHHHHHMSHMAPTHQLPPSDVRKIILELQPLSRGLLEDYQKKETGVPESNRTLLLCLTSDSQPPRLNSSAILPYFRAIRPLSDKNIIDKIIEQLDKLKFQHEPETEISVPADTFECKSFILTILQQFSACLESVFKSLNSGPQLQICAKYSSVTAWTPAAGRSCKMEGCRWWR

SEQ ID NO: 4 - protein, 164 aa, Artificial Sequence
  chimeric immunogen
MKHHHHHHMSHMAPTHQLPPSDVRKIILELQPLSRGLLEDYQKKETGVPESNRTLLLCLTSDSQPPRLNSSAILPYFRAIRPLSDKNIIDKIIEQLDKLKFQHEPETEISVPADTFECKSFILTILQQFSACLESVFKSLNSGPQLCFKRYELRLPAKRKRKRN

SEQ ID NO: 5 - protein, 175 aa, Artificial Sequence
  chimeric immunogen
MKHHHHHHMSHMAPTHQLPPSDVRKIILELQPLSRGLLEDYQKKETGVPESNRTLLLCLTSDSQPPRLNSSAILPYFRAIRPLSDKNIIDKIIEQLDKLKFQHEPETEISVPADTFECKSFILTILQQFSACLESVFKSLNSGPQVKSPQKSYLFPSSMIGIGSLPSCWACWIQQ

SEQ ID NO: 6 - protein, 182 aa, Artificial Sequence
  chimeric immunogen
MKHHHHHHMTCSLSFGAPISKEDLRTTIDLLKQESQDLYNNYSIKQASGMSADESIQLPCFSLDREALTNISVIIAHLEKVKVLSENTVDTSWVIRWLTNISCFNPLNLNISVPGNTDESYDCKVFVLTVLKQFSNCMAELQAKDNTTCLKIQKLQGKCSQPGMVGCSLTTWRTSMVLGRNI

SEQ ID NO: 7 - protein, 183 aa, Artificial Sequence
  chimeric immunogen
MKHHHHHHMLKIQKLQGKCSQPGMVGCSLTTWRTSMVLGRNIMTCSLSFGAPISKEDLRTTIDLLKQESQDLYNNYSIKQASGMSADESIQLPCFSLDREALTNISVIIAHLEKVKVLSENTVDTSWVIRWLTNISCFNPLNLNISVPGNTDESYDCKVFVLTVLKQFSNCMAELQAKDNTTC

SEQ ID NO: 8 - protein, 95 aa, Artificial Sequence
  Canonical insulin
MKHHHHHHMFVKQHLCGPHLVEALYLVCGERGFFYTPKSGGGFVKQHLCGSHLVEALYLVCGERGFFYTPMSGGGIVDQCCTSICSLYQLENYCN

SEQ ID NO: 9 - protein, 112 aa, Artificial Sequence
  chimeric immunogen
MKHHHHHHMFVKQHLCGPHLVEALYLVCGERGFFYTPKSGGGFVKQHLCGSHLVEALYLVCGERGFFYTPMSGGGIVDQCCTSICSLYQLENYCNFLISMPEKCVNTWIMKI

SEQ ID NO: 10 - protein, 110 aa, Artificial Sequence
  chimeric immunogen
MKHHHHHHMFVKQHLCGPHLVEALYLVCGERGFFYTPKSGGGFVKQHLCGSHLVEALYLVCGERGFFYTPMSGGGIVDQCCTSICSLYQLENYCNEFDIRRIRQMLIITK

SEQ ID NO: 11 - protein, 93 aa, Artificial Sequence
  IgE-CH3
MKHHHHHHMFIPPTVKLFHSSCNPVGDTHTTIQLLCLISGYVPGDMEVIWLVDGQKATNIFPYTAPGTKEGNVTSTHSELNITQGEWVSQKTY

SEQ ID NO: 12 - protein, 126 aa, Artificial Sequence
  IgE-CH3
MKHHHHHHMFIPPTVKLFHSSCNPVGDTHTTIQLLCLISGYVPGDMEVIWLVDGQKATNIFPYTAPGTKEGNVTSTHSELNITQGEWVSQKTYLKIQKLQGKCSQPGMVGCSLTTWRTSMVLGRNI

SEQ ID NO: 13 - protein, 176 aa, Artificial Sequence
  Canonical 5ES
MKHHHHHHMVYYHKNNKSWMESEFRVYSSANNCTFEYVSQPFLMDLEGKQGNFKNGGKRISNCVADYSVLYNSASFSTFKCYGVSPTKLNDLCGGSTEIYQAGSTPCNGVEGFNCYFPLQSYGFQPTGGVCGPKKSTNLVKNKCVNFNFGGDKNTQEVFAQVKQIYKTPPIKDFGG

SEQ ID NO: 14 - protein, 192 aa, Artificial Sequence
  chimeric immunogen
MKHHHHHHMVYYHKNNKSWMESEFRVYSSANNCTFEYVSQPFLMDLEGKQGNFKNGGKRISNCVADYSVLYNSASFSTFKCYGVSPTKLNDLCGGSTEIYQAGSTPCNGVEGFNCYFPLQSYGFQPTGGVCGPKKSTNLVKNKCVNFNFGGDKNTQEVFAQVKQIYKTPPIKDFGGPSGPSWASWLRCWCWS

SEQ ID NO: 15 - protein, 184 aa, Artificial Sequence
  chimeric immunogen
MVYYHKNNKSWMESEFRVYSSANNCTFEYVSQPFLMDLEGKQGNFKNGGKRISNCVADYSVLYNSASFSTFKCYGVSPTKLNDLCGGSTEIYQAGSTPCNGVEGFNCYFPLQSYGFQPTGGVCGPKKSTNLVKNKCVNFNFGGDKNTQEVFAQVKQIYKTPPIKDFGGPSGPSWASWLRCWCWS

SEQ ID NO: 16 - protein, 209 aa, Artificial Sequence
  chimeric immunogen
MKHHHHHHMVYYHKNNKSWMESEFRVYSSANNCTFEYVSQPFLMDLEGKQGNFKNGGKRISNCVADYSVLYNSASFSTFKCYGVSPTKLNDLCGGSTEIYQAGSTPCNGVEGFNCYFPLQSYGFQPTGGVCGPKKSTNLVKNKCVNFNFGGDKNTQEVFAQVKQIYKTPPIKDFGGLKIQKLQGKCSQPGMVGCSLTTWRTSMVLGRNI

SEQ ID NO: 17 - protein, 198 aa, Artificial Sequence
  chimeric immunogen
MKHHHHHHMVYYHKNNKSWMESEFRVYSSANNCTFEYVSQPFLMDLEGKQGNFKNGGKRISNCVADYSVLYNSASFSTFKCYGVSPTKLNDLCGGSTEIYQAGSTPCNGVEGFNCYFPLQSYGFQPTGGVCGPKKSTNLVKNKCVNFNFGGDKNTQEVFAQVKQIYKTPPIKDFGGSAKLSWTTFQILSWKPMFHFWY

SEQ ID NO: 18 - protein, 106 aa, Artificial Sequence
  Canonical Staphylococcus aureus protein
MKHHHHHHQLEKLNNDSKDKFNDIPKEQRAMITSEGAFKYFSKQYGITPGYIWEINTEKQGTPEQMRQAIEFVKKHKLKHLLVETSVDKKAMESLSEETKKDIFGE

SEQ ID NO: 19 - protein, 183 aa, Artificial Sequence
  Canonical Cryptosporidium parvum protein
MKHHHHHHSLTEETSETATVDLFAFTLNGGKRIEVAVPNAEETSKRDKYSLVADDSAFYTGKNSGSTDGVYKLNENGDLVDKDNKVLLKDAGSSGGSLSEETSEAAATVDLFAFTLDGGKRIEVAVPNVEDASKRDKYSLVADDKPFYTGANSGTTNGVYRLNENGDLVDKDNTVLLKDAGSS

SEQ ID NO: 20 - protein, 19 aa, Artificial Sequence
  TI segment
LCFKRYELRLPAKRKRKRN

SEQ ID NO: 21 - protein, 33 aa, Artificial Sequence
  TI segment
LKIQKLQGKCSQPGMVGCSLTTWRTSMVLGRNI

SEQ ID NO: 22 - protein, 30 aa, Artificial Sequence
  TI segment
VKSPQKSYLFPSSMIGIGSLPSCWACWIQQ

SEQ ID NO: 23 - protein, 16 aa, Artificial Sequence
  TI segment
PSGPSWASWLRCWCWS

SEQ ID NO: 24 - protein, 22 aa, Artificial Sequence
  TI segment
SAKLSWTTFQILSWKPMFHFWY

SEQ ID NO: 25 - protein, 15 aa, Artificial Sequence
  TI segment
EFDIRRIRQMLIITK

SEQ ID NO: 26 - protein, 30 aa, Artificial Sequence
  TI segment
LQICAKYSSVTAWTPAAGRSCKMEGCRWWR

SEQ ID NO: 27 - protein, 17 aa, Artificial Sequence
  TI segment
FLISMPEKCVNTWIMKI

SEQ ID NO: 28 - protein, 30 aa, Artificial Sequence
  TI segment
WRRWAAPWFWSSLQLGGLVFRGPGPRARSR

SEQ ID NO: 29 - protein, 19 aa, Artificial Sequence
  TI segment
WTKWRLSWPWKTNLGLKFL

SEQ ID NO: 30 - protein, 30 aa, Artificial Sequence
  TI segment
RFPARAPWRCRAPRSTCCIPATIRWPRAST

SEQ ID NO: 31 - protein, 19 aa, Artificial Sequence
  TI segment
HLKCKLKKFDRWDPIKRGQ

SEQ ID NO: 32 - protein, 27 aa, Artificial Sequence
  TI segment
LLCCFSAFPSFLLKDGRRFSSPGWWSC

SEQ ID NO: 33 - protein, 30 aa, Artificial Sequence
  TI segment
WSIWLSREQRIGLAVPWRRRWRAWGPILMP

SEQ ID NO: 34 - protein, 34 aa, Artificial Sequence
  TI segment
MLWMVQKAWLEARKYWILVHQSKFLLVLRLWAES

SEQ ID NO: 35 - protein, 30 aa, Artificial Sequence
  TI segment
LQICGKCSSVTAWTLAAGRSCKMEGCRWWK

SEQ ID NO: 36 - protein, 30 aa, Artificial Sequence
  TI segment
WRKRKRNWPRKQGRRLLTIWLLGKMNELGS

SEQ ID NO: 37 - protein, 23 aa, Artificial Sequence
  TI segment
LCAPRRSLLSVIGQKNLRNSTAK

SEQ ID NO: 38 - protein, 30 aa, Artificial Sequence
  TI segment
LTAPRAWRARTASPWTAATVASGRRKTRLT

SEQ ID NO: 39 - protein, 22 aa, Artificial Sequence
  TI segment
IPKDRLQHQQKLQWLMPYMKYQ

SEQ ID NO: 40 - protein, 22 aa, Artificial Sequence
  TI segment
MRSTLSGRDFHPCRWLMKSLAF

SEQ ID NO: 41 - protein, 26 aa, Artificial Sequence
  TI segment
LGLGRNGIRNHRNPETLQLKFVVIGK

SEQ ID NO: 42 - protein, 16 aa, Artificial Sequence
  TI segment
TLIPRGTRKHCIWVLS

SEQ ID NO: 43 - protein, 15 aa, Artificial Sequence
  TI segment
KIQKLQGKCSQPGMV

SEQ ID NO: 44 - protein, 30 aa, Artificial Sequence
  TI segment
QRKPRRRPRERALSCTRTLQIRKPHPVANL

SEQ ID NO: 45 - protein, 19 aa, Artificial Sequence
  TI segment
RCFKRCALRLPAKRRRKRN

SEQ ID NO: 46 - protein, 30 aa, Artificial Sequence
  TI segment
TWPRTSCGCERNCRRRCSRERKPKAPCSHS

SEQ ID NO: 47 - protein, 30 aa, Artificial Sequence
  TI segment
WRKKKRNWLRRQGRRLLTTWPPERMSEHAS

SEQ ID NO: 48 - protein, 11 aa, Artificial Sequence
  TI segment
HLKCKLKKSGR

SEQ ID NO: 49 - protein, 34 aa, Artificial Sequence
  TI segment
MLWMALKAWLEARKYWIQGHQSKFLLVLRPWAES

SEQ ID NO: 50 - protein, 20 aa, Artificial Sequence
  TI segment
FAKLSWTTYQILSWRPMSLY

SEQ ID NO: 51 - protein, 19 aa, Artificial Sequence
  Canonical peptide
ALLQKVRAEIASKEKEEEE

SEQ ID NO: 52 - protein, 170 aa, Artificial Sequence
  chimeric immunogen
MSHMAPTHQLPPSDVRKIILELQPLSRGLLEDYQKKETGVPESNRTLLLCLTSDSQPPRLNSSAILPYFRAIRPLSDKNIIDKIIEQLDKLKFQHEPETEISVPADTFECKSFILTILQQFSACLESVFKSLNSGPQLKIQKLQGKCSQPGMVGCSLTTWRTSMVLGRNI

SEQ ID NO: 53 - protein, 167 aa, Artificial Sequence
  chimeric immunogen
MSHMAPTHQLPPSDVRKIILELQPLSRGLLEDYQKKETGVPESNRTLLLCLTSDSQPPRLNSSAILPYFRAIRPLSDKNIIDKIIEQLDKLKFQHEPETEISVPADTFECKSFILTILQQFSACLESVFKSLNSGPQLQICAKYSSVTAWTPAAGRSCKMEGCRWWR

SEQ ID NO: 54 - protein, 156 aa, Artificial Sequence
  chimeric immunogen
MSHMAPTHQLPPSDVRKIILELQPLSRGLLEDYQKKETGVPESNRTLLLCLTSDSQPPRLNSSAILPYFRAIRPLSDKNIIDKIIEQLDKLKFQHEPETEISVPADTFECKSFILTILQQFSACLESVFKSLNSGPQLCFKRYELRLPAKRKRKRN

SEQ ID NO: 55 - protein, 167 aa, Artificial Sequence
  chimeric immunogen
MSHMAPTHQLPPSDVRKIILELQPLSRGLLEDYQKKETGVPESNRTLLLCLTSDSQPPRLNSSAILPYFRAIRPLSDKNIIDKIIEQLDKLKFQHEPETEISVPADTFECKSFILTILQQFSACLESVFKSLNSGPQVKSPQKSYLFPSSMIGIGSLPSCWACWIQQ

SEQ ID NO: 56 - protein, 174 aa, Artificial Sequence
  chimeric immunogen
MTCSLSFGAPISKEDLRTTIDLLKQESQDLYNNYSIKQASGMSADESIQLPCFSLDREALTNISVIIAHLEKVKVLSENTVDTSWVIRWLTNISCFNPLNLNISVPGNTDESYDCKVFVLTVLKQFSNCMAELQAKDNTTCLKIQKLQGKCSQPGMVGCSLTTWRTSMVLGRNI

SEQ ID NO: 57 - protein, 174 aa, Artificial Sequence
  chimeric immunogen
LKIQKLQGKCSQPGMVGCSLTTWRTSMVLGRNIMTCSLSFGAPISKEDLRTTIDLLKQESQDLYNNYSIKQASGMSADESIQLPCFSLDREALTNISVIIAHLEKVKVLSENTVDTSWVIRWLTNISCFNPLNLNISVPGNTDESYDCKVFVLTVLKQFSNCMAELQAKDNTTC

SEQ ID NO: 58 - protein, 87 aa, Artificial Sequence
  Canonical insulin
MFVKQHLCGPHLVEALYLVCGERGFFYTPKSGGGFVKQHLCGSHLVEALYLVCGERGFFYTPMSGGGIVDQCCTSICSLYQLENYCN

SEQ ID NO: 59 - protein, 104 aa, Artificial Sequence
  chimeric immunogen
MFVKQHLCGPHLVEALYLVCGERGFFYTPKSGGGFVKQHLCGSHLVEALYLVCGERGFFYTPMSGGGIVDQCCTSICSLYQLENYCNFLISMPEKCVNTWIMKI

SEQ ID NO: 60 - protein, 102 aa, Artificial Sequence
  chimeric immunogen
MFVKQHLCGPHLVEALYLVCGERGFFYTPKSGGGFVKQHLCGSHLVEALYLVCGERGFFYTPMSGGGIVDQCCTSICSLYQLENYCNEFDIRRIRQMLIITK

SEQ ID NO: 61 - protein, 85 aa, Artificial Sequence
  IgE-CH3
MFIPPTVKLFHSSCNPVGDTHTTIQLLCLISGYVPGDMEVIWLVDGQKATNIFPYTAPGTKEGNVTSTHSELNITQGEWVSQKTY

SEQ ID NO: 62 - protein, 118 aa, Artificial Sequence
  chimeric immunogen
MFIPPTVKLFHSSCNPVGDTHTTIQLLCLISGYVPGDMEVIWLVDGQKATNIFPYTAPGTKEGNVTSTHSELNITQGEWVSQKTYLKIQKLQGKCSQPGMVGCSLTTWRTSMVLGRNI

SEQ ID NO: 63 - protein, 168 aa, Artificial Sequence
  Canonical 5ES
MVYYHKNNKSWMESEFRVYSSANNCTFEYVSQPFLMDLEGKQGNFKNGGKRISNCVADYSVLYNSASFSTFKCYGVSPTKLNDLCGGSTEIYQAGSTPCNGVEGFNCYFPLQSYGFQPTGGVCGPKKSTNLVKNKCVNFNFGGDKNTQEVFAQVKQIYKTPPIKDFGG

SEQ ID NO: 64 - protein, 184 aa, Artificial Sequence; identical to SEQ ID NO: 15
  chimeric immunogen

SEQ ID NO: 65 - protein, 198 aa, Artificial Sequence
  chimeric immunogen
MVYYHKNNKSWMESEFRVYSSANNCTFEYVSQPFLMDLEGKQGNFKNGGKRISNCVADYSVLYNSASFSTFKCYGVSPTKLNDLCGGSTEIYQAGSTPCNGVEGFNCYFPLQSYGFQPTGGVCGPKKSTNLVKNKCVNFNFGGDKNTQEVFAQVKQIYKTPPIKDFGGVKSPQKSYLFPSSMIGIGSLPSCWACWIQQ

SEQ ID NO: 66 - protein, 201 aa, Artificial Sequence
  chimeric immunogen
MVYYHKNNKSWMESEFRVYSSANNCTFEYVSQPFLMDLEGKQGNFKNGGKRISNCVADYSVLYNSASFSTFKCYGVSPTKLNDLCGGSTEIYQAGSTPCNGVEGFNCYFPLQSYGFQPTGGVCGPKKSTNLVKNKCVNFNFGGDKNTQEVFAQVKQIYKTPPIKDFGGLKIQKLQGKCSQPGMVGCSLTTWRTSMVLGRNI

SEQ ID NO: 67 - protein, 190 aa, Artificial Sequence
  chimeric immunogen
MVYYHKNNKSWMESEFRVYSSANNCTFEYVSQPFLMDLEGKQGNFKNGGKRISNCVADYSVLYNSASFSTFKCYGVSPTKLNDLCGGSTEIYQAGSTPCNGVEGFNCYFPLQSYGFQPTGGVCGPKKSTNLVKNKCVNFNFGGDKNTQEVFAQVKQIYKTPPIKDFGGSAKLSWTTFQILSWKPMFHFWY

SEQ ID NO: 68 - protein, 98 aa, Artificial Sequence
  Canonical Staphylococcus aureus protein
QLEKLNNDSKDKFNDIPKEQRAMITSEGAFKYFSKQYGITPGYIWEINTEKQGTPEQMRQAIEFVKKHKLKHLLVETSVDKKAMESLSEETKKDIFGE

SEQ ID NO: 69 - protein, 175 aa, Artificial Sequence
  Canonical  Cryptosporidium parvum protein
SLTEETSETATVDLFAFTLNGGKRIEVAVPNAEETSKRDKYSLVADDSAFYTGKNSGSTDGVYKLNENGDLVDKDNKVLLKDAGSSGGSLSEETSEAAATVDLFAFTLDGGKRIEVAVPNVEDASKRDKYSLVADDKPFYTGANSGTTNGVYRLNENGDLVDKDNTVLLKDAGSS

SEQ ID NO: 70 - protein, 137 aa, Artificial Sequence
  Canonical IL31
MSHMAPTHQLPPSDVRKIILELQPLSRGLLEDYQKKETGVPESNRTLLLCLTSDSQPPRLNSSAILPYFRAIRPLSDKNIIDKIIEQLDKLKFQHEPETEISVPADTFECKSFILTILQQFSACLESVFKSLNSGPQ